European Patent Specification EP 3 914 728 B1, published April 5, 2023. Title: OLIGONUCLEOTIDES ASSOCIATED WITH ANTIBODIES. Applicant: Cellular Research, Inc. Shum, Eleen Lazaruk, Katherine Prosen, Dennis E. Jensen, Devon Rosenfeld, David Lai, Janice H. Ghadiali, James Chang, Christina. The sequence listing filed with the application follows.

SEQUENCE LISTING (8 sequences)

SEQ ID NO: 1 - DNA, 95 bp, Artificial Sequence
  Synthetic Oligonucleotide
  5'AmMC6 (1)..(1): 5' Amino Modifier C6
gttgtcaagatgctaccgttcagagtacgtggagttggtggcccgaccccgagcgctacgagccccccggaaaaaaaaaaaaaaaaaaaaaaaaa

SEQ ID NO: 2 - DNA, 200 bp, Artificial Sequence
  Synthetic Oligonucleotide
  5AmMC6 (1)..(1): 5' Amino Modifier C6
gttgtcaagatgctaccgttcagagctactgtccgaagttaccgtgtatctaccacgggtggtttttcgaatccggaaaagatagtaataagtgttttagttggaataagtcgcaacttttggagacggttacctctcaatttttctgatccgtaggccccccgatctcggcctcaaaaaaaaaaaaaaaaaaaaaaaaa

SEQ ID NO: 3 - DNA, 25 bp, Artificial Sequence
  Synthetic Oligonucleotide
gttgtcaagatgctaccgttcagag

SEQ ID NO: 4 - DNA, 20 bp, Artificial Sequence
  Synthetic Oligonucleotide
acacgacgctcttccgatct

SEQ ID NO: 5 - DNA, 95 bp, Artificial Sequence
  Synthetic Oligonucleotide
gttgtcaagatgctaccgttcagagccccatgtctagtacctattggtcccctatcctcagattcgtttaaaaaaaaaaaaaaaaaaaaaaaaaa

SEQ ID NO: 6 - DNA, 26 bp, Artificial Sequence
  Synthetic Oligonucleotide
tttttttttttttttttttttttttt

SEQ ID NO: 7 - DNA, 95 bp, Artificial Sequence
  Synthetic Oligonucleotide
  5AmMC6 (1)..(1): 5' Amino Modifier C6
gttgtcaagatgctaccgttcagagattcaagggcagccgcgtcacgattggatacgactgttggaccggaaaaaaaaaaaaaaaaaaaaaaaaa

SEQ ID NO: 8 - DNA, 102 bp, Artificial Sequence
  Synthetic Oligonucleotide
  5'AmMC12 (1)..(1): 5' Amino Modifier C12
  misc_feature (24)..(25): n is a, c, g, or t
  misc_feature (27)..(30): n is a, c, g, or t
  misc_feature (32)..(33): n is a, c, g, or t
  misc_feature (35)..(75): n is a, c, g, or t
cagacgtgtgctcttccgatctvnnvnnnnvnnvnnnnnnnnnnnnnnnnnnnnnnnnnnnnnnnnnnnnnnnnnbbaaaaaaaaaaaaaaaaaaaaaaaaa